European Patent Specification EP 4 086 351 B1, published December 11, 2024. Title: VIRAL VECTORS FOR TREATING NEUROGENIC DETRUSOR OVERACTIVITY. Applicant: UNIVERSITE DE VERSAILLES-ST QUENTIN EN YVELINES ASSISTANCE PUBLIQUE - HOPITAUX DE PARIS. The sequence listing filed with the application follows.

SEQUENCE LISTING (33 sequences)

SEQ ID NO: 1 - DNA, 1020 bp, rat
atatggagaggtggggtgaggggtggcagagagggatcgagagaggagagaggggaaccagatgtagcagccaggaggccaaaggtacaaaaggggtgggtaaccaaaatgtctggattatataaaaaagagccagaggtcaggcccactttgatatgttaaataggcacctcagccatttatccaggtttgaaatgtaatataatttacatccccctggcttcctagagaccgttgtttagacggatgacctctgcagaatgtttgagggtgcagtcttgcatgtactccctggtgggctttcttgggcaggatctgggcaggaatgggcttgttctagtcacccactgcgtatgatggatgaacccgcttcctagtagttaggatggcactgggggaggcgagaaattagcacacgtaacgttttcttgtgttctattgttcactaagggaccccagtcaagcaagactgggccttggaagacctagagaccaccaaacctaatctctaccccgggtctgagtacacagggactcagagtcccaaagggggcagggcctccagacaggtggctcagaggtcccagtcctttggaaacatggcatcttcaggacactgggctttgcatctctggctgtgacagtcctttaagggagctactcctcagacatacaggagagatggtttggaaagtccgagatccaaagcctggttcaggctggactgggctgcaggctgctaagtgctcctctgccctggcatggctgggggtggggcattggctgtggtttctgaaaaagggcaaaaatgatgggaaaagctttgggatcctctgggaatcggagccgtggtaacagcagctgctgccattgctgcaaatgtttccttgagtgccagagtatgcccagagcccatccctgccgtacgccaggggaggggcgaggaccctcacagaggcagggaggccggccactcttaccacacagcagcctggctctcccacaaagaacagctatgca

SEQ ID NO: 2 - DNA, 975 bp, human
gacttaccaggagctagggcatttataagcattgtgccctgaagataagttcaccccaggcagttctgaaaaggactcgtcaaacatgtcctgctgtagaataatttctaaaaatgtttttcagatcttaggagtaatataaacatgcagaaaagtagaaggaagaaaataatgacctgatacaaactaaaggtttgagtgctgtgtgaacagtctaagggaggttattgaattggggtgaaaagaatagaaagaagagcgcagataattgtaatagtaacaatagctaatatttattgaagctttcccatgctgggcacaggttcaagtgctttacaggggtcgcctcatttaattattactcatttctgtgtaggtgtgtagccggtgggctagttcaggttcttgactttgggacagaaaataatttgaaagtgagtcaaaagcaaaagcaagcaagagagttgactgcaaagccaaagtacactctagcagccggtcagaacgggccactcaaaggcaagacagctctgtctaatactgggggatctccctttatgggaaatttgcatgattattcatgaaggggtggtaaggggtgttgctattaagcatgttaggagtggtttcttaggtccacatgtgcagtggctgtacatgctagtacatccatcgcatgtcttataagcattttaaatctccacctgggggtgtgttttttactattataatgagcacaggtcagcccaaggacactaatcacgggtttctgtgcttgtacaaatgtggggatttttctcttctgctcctgcctttttgctgtagggtgttctaaccacgagctcaggatgcggtctgtgcactgttaggtggtttgttctcttcatcaatttgacaagtttcttgtttcctgtcaagggaggctctgaccacctcatctaacctgcctcaggtgcagccttattgccattttac

SEQ ID NO: 3 - DNA, 1360 bp, rat
gagggacttgaaggcaggcttgggacaatttgagaatgaacccctaaggatgcttctgtgggccacagagactgctgagtggctgtgctttctggatacggtaccattttggaaagagaggagagtctctgtgccaggagaagtgtgactggtagtgaatgtgaggtttagtacggggcaacatctccacagcgctgtcaagcctgcctgcctgctcttcagctctttagctcggagatctaagggtgggggtaggaggggagccaccggaccaaatacaactgggacatcttggcaaacagcagcgggaagcaaaggggcagctgtgcaaatccttaggcaggcgggcgggcgggcaggcgggcgggcgggcgggcaggcgggcaggcgggcgggcaggcggccggatgagtagtgatggatagccaggcaggaggtggagagatctacactggagactttagaggcatctggtccttcctcacactgtccccactaccccgtacccctactccctaccccaagcaggacccagctgaatacaaccccttctcacacatgtgagtgagtgagttatccagcacataagaatgccaagctgaagacggatgattcactttggggaaggagagattttatagctcaggaaacaccaaggtttctgcctactagccaggcccttcaaaaggggaccaggatacccactgaaaagtttaatatgttgagctttcgtgcaggcctttgggggtttgggggggggggaattttgaattttttttttcgttttgtttttacctgtggtcacataaccagcacgaggcagctacaaggttcaggtctgacagagcccctgtgtccagcaccaacacctttggctatcagcctaaacctgtgccaccctgccaaagccagccttgcagaccaagagtccacccctacggtgcactaaagtcttccggattaggcacggactagggtcggggcacgattagaatcagacatgcagcaaggagtacttgagatactggactctactctccaaggtccagagattggagtcggggatgttcaaagtcaggagggaagaagagataaaatttaccttgacgtcaaaaggccctccaaattcccgctaattttaagggtggttctcactgctccccaccatcctcccacttccatcaatgacctcaatttaaattcaaatggtgtcatcttgctagatgctcggagttctggaagcaccgaggtgacgcaatctgtctggggcacggggcccttccacctattggctgcctggcgccccgggacccctcccaactaccgcggcgggaataagagcagctgcaggcgcttggaa

SEQ ID NO: 4 - DNA, 1837 bp, human
gatcaattaagggcatcttagaagttaggcgttcccgctgcctcctttgagcacggaggccaccaaccccctagggggaagagatgtagcgcgaggcaggggtgtcgtgctaagaaatttcgacgcttctggggactgaggacaaaggtgcggacacgaccccggggtacctggagttccgtgactcgcgccacggacggcacacctaggggctaatttctgctctgcctcaaagaacctcaagctagagtccttgcctccgcccacagccccgggatgccgctgctgcgctcaccgcacaggcagcgcccggaccggctgcagcagatcgcgcgctgcgcgttccaccgggagatggtggagacgctgaaaagcttctttcttgccactctggacgctgtgggcggcaagcgccttagtccctacctctgctgagctgaacgctcaggcacagtggaactgaaacccggttctgcgggatgtgagagctgttgaggtcacgcgtaattgggtgtgatggagggcgcctgttcgtgatgtgtgcaggtttgatgcaagcaggtcatcgtcgtgcgagtgtgtggatgcgaccgcccgagagactcggaggcaggcttgggacacgtttgagtgaacacctcaggatactcttctggccagtatctgttttttagtgtctgtgattcagagtgggcacatgttgggagacagtaatgggtttgggtgtgtgtaaatgagtgtgaccggaagcgagtgtgagcttgatctaggcagggaccacacagcactgtcacacctgcctgctctttagtagaggactgaagtgcgggggtgggggtacggggccggaatagaatgtctctgggacatcttggcaaacagcagccggaagcaaaggggcagctgtgcaaacggctcaggcaggtgatggatggcagggtaggaagggggaggtccagaggtctggatggaggcttccgcatctgtaccttgcaactcacccctcaggcccagcaggtcatcggccccctcctcacacatgtaatggatctgaagagtaccccgggacagtccggggagatggagattcggaaagtatccatggagatcttacagaatcccctatgcggaccaggaaactcttgtagatccctgcctatctgaggcccaggcgctgggctgtttctcacaatattccttcaagatgagattgtggtccccatttcaaagatgagtacactgagcctctgtgaagttacttgcccatgatcacacaaccaggaattgggccaactgtaattgaactcctgtctaacaaagttcttgctcccagctccgtctcttgtttcccacgagccctggccctctgtgggtaataccagctactggagtcagatttcttgggcccagaacccacccttaggggcattaacctttaaaatctcacttgggcaggggtctgggatcagagttggaagagtccctacaatcctggaccctttccgccaaatcgtgaaaccaggggtggagtggggcgagggttcaaaaccaggccggactgagaggtgaaattcaccatgacgtcaaactgccctcaaattcccgctcactttaagggcgttacttgttggtgcccccaccatcccccaccatttccatcaatgacctcaatgcaaatacaagtgggacggtcctgctggatcctccaggttctggaagcatgagggtgacgcaacccaggggcaaaggacccctccgcccattggttgctgtgcactggcggaactttcccgacccacagcggcgggaataagagcagtcgctggcgctgggaggc

SEQ ID NO: 5 - DNA, 1633 bp, rat
tggccctgccctgccctgttcagaggcttcttggcagtgcggcccatttgtgctgtcctgcatccagtgtatcagcctagctaagtgtgagccatttccatttggggctactcttcagttccttttttaaaatagcttagccctctcccttacctctacccctagacagggtttcatgaattccaagcaggggcctcaactcacatttagccaggaatgatcttgaactgacctcctgagtgctggggttacaggtgtgatcaccttgctgctttaggaggtgctgggaacaacccagggcatcgtgtgtgttaagcacacactcccagctaagctacatccccagtccctctttctagaaaacatcattagttaaatatattcaggggagaagaggtcacaggtctggccagctgccccatcctttagtgcagggtcagctcccagaactgctctgctctgctctgcaagctggtgattctccttacctgtgattactccagatctgcctatttccaagatgccatttgaaggggaggggtctgcttcccactgtgactgggctatgggatccttgaccaccttgcttcatgatttgatacatttgttgtattcaaaaacttgaactgtaggatgccattaagagtctgtttatatttttggaatatttgtattacaattgttttaataaaggccggtttaaaaacctatgcatgagtgggggctgctttccttccccgccactggtcccacacacggtggacgctgttcttcccgtattccctttttggtcctaagattatagcacccagcagaacaaacactgggttctgatcaaggttgcaaaggttggactgcattagctcttctctggcccaggttggaaccaactccctctcccctgggtacttagcaaacatgtgcttgctgtgctattgactgctgggtatagactgaagcccttggggaattggggactcctgtgcatgctcttgatactgccaaacaggagccatgagactcagagcccagcacggtttccaggcacatagtaggaggacttgtaaagactaaacaaaagctttcctatcaccacaaatttgcccagaatcatctcgccatcctgaacatccaggcatacagtaggagagctctagccagccgcctgtcatcagcataatacattcatatctacaatatggcaaattcatatcctccctcactgaattattgatggactctgcacttttaaaaaaatcaatagaccaggggtggagctggagttaaaagaagcctttaaaagtctgctcttcttgtttttgctgttttgaataggagcagataaagctttccccgctggtttgaataagtcaagcccagggctaggtcggctgtgattggccagagctgggaaaatgtggttatgatgcaaacgcaagcaaatataacccagtgtctgtgtgctgtgtggccattgctgaaacaggcttcaggacccgaggtcgcctgcttcgggaccgctcgtcagtacttcacctgctgctttgctgggaaagggagaacagagggtcaggtaaggtctactgtgtgtgtccttgtcagctgaaggtgaggggacaggggtcacgccttc

SEQ ID NO: 6 - DNA, 1460 bp, human
gcagcacagggtggggcagcacaagttatcaaattaaattctcaaacactggctgctccgcaccattgccttgctttagtcctgctacagcagtagacaaagcgagtctgctttgagctttatggttttttgccaaagtccatactagatggcgcatgctctccaaacttggctttgtccatcaaggttcaagaaaacaatggtcagacatgttcctcttaacaaacagtatgtccccaaacagcaaaaatgcatacagtcctttctgggtgaatttttaaatcttacataaatccatcaaccccatcctttttcctttgcctcttgggagaaattaatctagctttacattaattatgcatgttatcagatttcaagctccttgagagcaggtattttaattctataaagcctctacgtggccttggacatgggtaggtgcttaattacccaagatgctccttgaatacagatggtacacgacctacacagacttagatctttaccacttcccccctctccccaccctgacttgctcaatcctgaaggaactggagacgtctaagtgtctgaggttcacgcttccacacagaagcttgggtctgtgtgggagggaaaaaggaagccatctgtccgcaggccagaccaggccacaccctgctagcacccagaaccctttgtcccaggcccagccctgccattttactttccttgcatctggaaagcacagggaatatagtagtgacaaaagaaggaagggttgtttgagtttaagaatagtttactctaaaaaaaaaaaaaaaaaaaaaaaaaggacaaaagccaaagagaaggtcaaagttgactgtggagaaggccttgcaagcagggaacttgggaagaattggaatgagagtgagagaaggcaactgagtttggaaatattttttctgactagcttttctttccaaatgccactgaacttagattggtttaggaagggttgtagtacatcaaagtggctagaagcacaggtttggggatcagataaggatttcattctagagtgtgatcttgtacaagttattcagcctttgcaaacctcagattcacacaatgtaagatgaagaaactcaccttctgaaaattagagataacatatgcaaagtgaatcaatacagggcttaacatatttatcacccctttggtaaataaccatgacgattaccagagctcttaagggcaatggcaggtgggaagcagaactcatgggtggtaatccccaggccagccaggctcaccatgtgcacttggacaagtccttgcccccatcattgtgaaatggtgcagggatgcaccatgagggtgtggcaggatggctgacaacagactgggaagcagctcggcagaaaaactggattgatgcccactatggcaagagatatcatctcccctcttgttctgtgatgtttcagtcctgg

SEQ ID NO: 7 - DNA, 351 bp, artificial
  VAMP2 Antisense
ttaagtgctgaagtaaactatgatgatgatgaggatgatggcgcaaatcactcccaagatgatcatcatcttgaggtttttccaccagtatttgcgcttgagcttggctgcgcttgtttcaaactgggaggcccccgcctggagtgcatctgcacggtcgtccagctccgacagcttctggtctcgctccaggaccttgtccacgttcaccctcatgatgtccaccacctcatccacctgggcctgggtctgctgcagtctcctgttactggtgaggtttggagggggtgcagggggaccaccctccccagccggggcagcagggggggccgtggcagcggtagcagacat

SEQ ID NO: 8 - DNA, 621 bp, artificial
  SNAP25 Antisense
ttaaccacttcccagcatctttgttgcacgttggttggcctcatcaattctggttttgttggaatcagccttctccatgatcctgtcgatctggcgattctgtgtatcgatctcattgcccatatccagggccatgtgacggaggttcccgatgatgccgctcacctgctctaggttttcatccatttcattttctcgggcatcatttgttaccctgcggatgaagccgccactgatggccatctgctcccgttcgtccactacacgagcaggctggctggccaccactccgtcctgattattgccccaggcttttttgtaagcatcacttgatttaagcttgttacaaggacatatgaaaaggccacagcatttccctaaatcttttaaatttttctcagcctccttcatgtcttggttgatatggttcatgccttcttcgacacgatcgagttgttctccttgttcatccaacataaccaaagtcctgataccagcatctttactctcttcaaccagttgcagcatacgacgggtgctttccagcgactcatcagccaactggtcagcccttcgctgcatctcctccagctcattgcgcatgtctgcgtcttcggccat

SEQ ID NO: 9 - DNA, 840 bp, artificial
  STX Antisense
ttaattcaggccaacggaaagtccaataatcaatgctaaaatgcccagcaacacaactactagcacaatgataattatcaatttcttccgggcctgactctggtatttcacagcttttttgctttcatctcgtgccttctccacgtggtccactgtgtgcatgacattcaactctatgttatctaacatctcaccctgattctccaccagcatggcgatgtccataaacatgtcgtgaagctccttgatgctgctctccagcctcacaatgtccttgtgtcgtccctcaatctcactgagggcttgcttggaaatctgtgagtcaatgatcccagaagtgaagatggccgggttgccactctccaacatctcctccagctcctcatcggttgtctttttgccagtaatttcgagctgccgctggattcgccctttgctgcgttctcggaagtccacttgagcttcattgtatttggtcatcacctccacaaacttccgagaaaggacagagtgctgggatttccgaatccgaaggtctgccgatgacctgacctcatcttcttcaatatgcttctccatgctcttcagtttgttccggacgttgttggcccttttcttaatctcagtgctgagctgctctaggtcatccttggtttttggctctggaatcggtgcagagagaatgatactgtagagtttcttagcctcctctacatgttctgagatcttgtcaatgttaagccgagtttcctcaatctcagaaaagaactcgtccataaaagccgtgttgtcgatagcaatctcaaccgcatcagtatcatcatcctgtgtcagttgcat

SEQ ID NO: 10 - protein, 457 aa, bacteria
MHHHHHHQFVNKQFNYKDPVNGVDIAYIKIPNVGQMQPVKAFKIHNKIWVIPERDTFTNPEEGDLNPPPEAKQVPVSYYDSTYLSTDNEKDNYLKGVTKLFERIYSTDLGRMLLTSIVRGIPFWGGSTIDTELKVIDTNCINVIQPDGSYRSEELNLVIIGPSADIIQFECKSFGHEVLNLTRNGYGSTQYIRFSPDFTFGFEESLEVDTNPLLGAGKFATDPAVTLAHELIHAGHRLYGIAINPNRVFKVNTNAYYEMSGLEVSFEELRTFGGHDAKFIDSLQENEFRLYYYNKFKDIASTLNKAKSIVGTTASLQYMKNVFKEKYLLSEDTSGKFSVDKLKFDKLYKMLTEIYTEDNFVKFFKVLNRKTYLNFDKAVFKINIVPKVNYTIYDGFNLRNTNLAANFNGQNTEINNMNFTKLKNFTGLFEFYKLLCVRGIITSKTKSLDKGYNKALN

SEQ ID NO: 11 - DNA, 1374 bp, bacteria
atgcaccaccaccaccaccaccagttcgtgaacaagcagttcaactacaaggaccccgtgaacggcgtggacatcgcctacatcaagatccccaacgtgggccagatgcagcccgtgaaggccttcaagatccacaacaagatctgggtgatccccgagagagacaccttcaccaaccccgaggagggcgacctgaaccccccccccgaggccaagcaggtgcccgtgagctactacgacagcacctacctgagcaccgacaacgagaaggacaactacctgaagggcgtgaccaagctgttcgagagaatctacagcaccgacctgggcagaatgctgctgaccagcatcgtgagaggcatccccttctggggcggcagcaccatcgacaccgagctgaaggtgatcgacaccaactgcatcaacgtgatccagcccgacggcagctacagaagcgaggagctgaacctggtgatcatcggccccagcgccgacatcatccagttcgagtgcaagagcttcggccacgaggtgctgaacctgaccagaaacggctacggcagcacccagtacatcagattcagccccgacttcaccttcggcttcgaggagagcctggaggtggacaccaaccccctgctgggcgccggcaagttcgccaccgaccccgccgtgaccctggcccacgagctgatccacgccggccacagactgtacggcatcgccatcaaccccaacagagtgttcaaggtgaacaccaacgcctactacgagatgagcggcctggaggtgagcttcgaggagctgagaaccttcggcggccacgacgccaagttcatcgacagcctgcaggagaacgagttcagactgtactactacaacaagttcaaggacatcgccagcaccctgaacaaggccaagagcatcgtgggcaccaccgccagcctgcagtacatgaagaacgtgttcaaggagaagtacctgctgagcgaggacaccagcggcaagttcagcgtggacaagctgaagttcgacaagctgtacaagatgctgaccgagatctacaccgaggacaacttcgtgaagttcttcaaggtgctgaacagaaagacctacctgaacttcgacaaggccgtgttcaagatcaacatcgtgcccaaggtgaactacaccatctacgacggcttcaacctgagaaacaccaacctggccgccaacttcaacggccagaacaccgagatcaacaacatgaacttcaccaagctgaagaacttcaccggcctgttcgagttctacaagctgctgtgcgtgagaggcatcatcaccagcaagaccaagagcctggacaagggctacaacaaggccctgaactga

SEQ ID NO: 12 - protein, 447 aa, bacteria
MHHHHHHPVTINNFNYNDPIDNNNIIMMEPPFARGTGRYYKAFKITDRIWIIPERYTFGYKPEDFNKSSGIFNRDVCEYYDPDYLNTNDKKNIFLQTMIKLFNRIKSKPLGEKLLEMIINGIPYLGDRRVPLEEFNTNIASVTVNKLISNPGEVERKKGIFANLIIFGPGPVLNENETIDIGIQNHFASREGFGGIMQMKFCPEYVSVFNNVQENKGASIFNRRGYFSDPALILMHELIHVLHGLYGIKVDDLPIVPNEKKFFMQSTDAIQAEELYTFGGQDPSIITPSTDKSIYDKVLQNFRGIVDRLNKVLVCISDPNININIYKNKFKDKYKFVEDSEGKYSIDVESFDKLYKSLMFGFTETNIAENYKIKTRASYFSDSLPPVKIKNLLDNEIYTIEEGFNISDKDMEKEYRGQNKAINKQAYEEISKEHLAVYKIQMCKSVK

SEQ ID NO: 13 - DNA, 1344 bp, bacteria
atgcaccaccatcatcaccaccctgttaccatcaataactttaactataacgatccaatagacaacaacaacatcatcatgatggagcccccctttgctagagggactggtcggtactacaaagcttttaagatcaccgatcggatttggattatccctgaacggtatacatttggctacaaacccgaagacttcaataaatcttctggtattttcaatcgagacgtgtgtgaatactatgatcccgactacctcaacactaacgataaaaagaacattttcctgcagacaatgattaagctgttcaatcggatcaagagtaaacccttgggtgaaaaacttctggagatgattatcaacggtataccttacctgggcgacaggagggtgccactcgaagagttcaatacaaacatagccagcgtgaccgtgaataagctgatcagtaacccaggcgaagttgagcggaagaagggaattttcgctaacctcatcatcttcggaccaggacctgtccttaacgagaatgagacaattgatattggaatccagaaccatttcgcatcacgcgaaggcttcgggggtatcatgcagatgaagttctgcccggagtatgtctctgtgttcaacaacgtgcaggaaaataagggagcgagcattttcaatcgcagaggctatttttccgaccccgcgctcatccttatgcacgagctgatccatgtcctgcacggactgtacggcatcaaagtcgacgatttgccaattgtgcccaacgaaaagaagttcttcatgcagtccaccgacgctatccaagcggaggagctctatacttttggcggacaggacccttctatcatcactccatctacagataagagtatatacgataaggttctccagaatttccgcggaatcgtcgaccgccttaacaaggtgctggtttgtatttccgacccaaacatcaatataaatatctataagaacaagttcaaagataaatataagttcgtggaggacagcgagggtaagtactctattgatgtggagagctttgataaactgtacaagtctctcatgttcggtttcacagagactaatatcgccgagaactataagataaaaacccgggcaagctatttctccgatagcctgccaccggttaagattaagaacctgctggacaatgaaatatataccatcgaggaaggatttaacatctccgacaaggacatggagaaagaataccggggacagaacaaggccattaataagcaggcttacgaggagattagcaaggagcacctggctgtgtacaaaatccagatgtgcaagtcagtgaagtag

SEQ ID NO: 14 - protein, 457 aa, bacteria
MHHHHHHPITINNFNYSDPVDNKNILYLDTHLNTLANEPEKAFRITGNIWVIPDRFSRNSNPNLNKPPRVTSPKSGYYDPNYLSTDSDKDPFLKEIIKLFKRINSREIGEELIYRLSTDIPFPGNNNTPINTFDFDVDFNSVDVKTRQGNNWVKTGSINPSVIITGPRENIIDPETSTFKLTNNTFAAQEGFGALSIISISPRFMLTYSNATNDVGEGRFSKSEFCMDPILILMHELNHAMHNLYGIAIPNDQTISSVTSNIFYSQYNVKLEYAEIYAFGGPTIDLIPKSARKYFEEKALDYYRSIAKRLNSITTANPSSFNKYIGEYKQKLIRKYRFVVESSGEVTVNRNKFVELYNELTQIFTEFNYAKIYNVQNRKIYLSNVYTPVTANILDDNVYDIQNGFNIPKSNLNVLFMGQNLSRNPALRKVNPENMLYLFTKFCHKAIDGRSLYNKTL

SEQ ID NO: 15 - DNA, 1374 bp, bacteria
atgcaccaccaccaccaccaccccatcaccatcaacaacttcaactacagcgaccccgtggacaacaagaacatcctgtacctggacacccacctgaacaccctggccaacgagcccgagaaggccttcagaatcaccggcaacatctgggtgatccccgacagattcagcagaaacagcaaccccaacctgaacaagccccccagagtgaccagccccaagagcggctactacgaccccaactacctgagcaccgacagcgacaaggaccccttcctgaaggagatcatcaagctgttcaagagaatcaacagcagagagatcggcgaggagctgatctacagactgagcaccgacatccccttccccggcaacaacaacacccccatcaacaccttcgacttcgacgtggacttcaacagcgtggacgtgaagaccagacagggcaacaactgggtgaagaccggcagcatcaaccccagcgtgatcatcaccggccccagagagaacatcatcgaccccgagaccagcaccttcaagctgaccaacaacaccttcgccgcccaggagggcttcggcgccctgagcatcatcagcatcagccccagattcatgctgacctacagcaacgccaccaacgacgtgggcgagggcagattcagcaagagcgagttctgcatggaccccatcctgatcctgatgcacgagctgaaccacgccatgcacaacctgtacggcatcgccatccccaacgaccagaccatcagcagcgtgaccagcaacatcttctacagccagtacaacgtgaagctggagtacgccgagatctacgccttcggcggccccaccatcgacctgatccccaagagcgccagaaagtacttcgaggagaaggccctggactactacagaagcatcgccaagagactgaacagcatcaccaccgccaaccccagcagcttcaacaagtacatcggcgagtacaagcagaagctgatcagaaagtacagattcgtggtggagagcagcggcgaggtgaccgtgaacagaaacaagttcgtggagctgtacaacgagctgacccagatcttcaccgagttcaactacgccaagatctacaacgtgcagaacagaaagatctacctgagcaacgtgtacacccccgtgaccgccaacatcctggacgacaacgtgtacgacatccagaacggcttcaacatccccaagagcaacctgaacgtgctgttcatgggccagaacctgagcagaaaccccgccctgagaaaggtgaaccccgagaacatgctgtacctgttcaccaagttctgccacaaggccatcgacggcagaagcctgtacaacaagaccctgtga

SEQ ID NO: 16 - protein, 429 aa, bacteria
MHHHHHHPKINSFNYNDPVNDRTILYIKPGGCQEFYKSFNIMKNIWIIPERNVIGTTPQDFHPPTSLKNGDSSYYDPNYLQSDEEKDRFLKIVTKIFNRINNNLSGGILLEELSKANPYLGNDNTPDNQFHIGDASAVEIKFSNGSQHILLPNVIIMGAEPDLFETNSSNISLRNNYMPSNHGFGSIAIVTFSPEYSFRFNDNSINEFIQDPALTLMHELIHSLHGLYGAKGITTTCIITQQQNPLITNRKGINIEEFLTFGGNDLNIITVAQYNDIYTNLLNDYRKIASKLSKVQVSNPQLNPYKDIFQEKYGLDKDASGIYSVNINKFDDILKKLYSFTEFDLATKFQVKCRETYIGQYKYFKLSNLLNDSIYNISEGYNINNLKVNFRGQNANLNPRIIKPITGRGLVKKIIRFCKNIVSVKGIRK

SEQ ID NO: 17 - DNA, 1290 bp, bacteria
atgcaccatcaccatcaccatcccaagattaattctttcaactataatgatccagtcaacgacaggaccattctctacatcaagccgggcggctgtcaggaattctacaaatcatttaacatcatgaagaatatttggatcatacctgaaagaaatgtgattggaaccacaccccaggatttccaccccccaacaagcttgaaaaacggagacagttcctactatgaccctaattatcttcagagcgatgaggagaaagacagattcctgaagatcgtgaccaaaatcttcaaccggatcaacaataatctctccgggggtattttgctggaggagctgtcaaaggcgaatccttaccttggcaatgataacacaccggacaatcagttccacataggagatgcttcagctgtcgagattaaattcagcaacggttcccagcatattctgcttccgaatgtcattattatgggagccgagccagacctgttcgagaccaattcttccaacataagcttgaggaataattacatgccatctaaccacggttttgggtcaatcgcaattgtcacttttagtccggagtacagcttccgctttaatgacaacagcatcaatgaattcatacaggatcccgctctgacactcatgcatgagctgatccactctctgcatggcctgtatggtgctaaggggatcaccaccacatgtattatcacgcagcagcaaaatccactgattacaaacaggaaaggcataaatattgaagagttcctgacattcggcggcaatgaccttaacattatcactgtggctcagtataacgatatttatactaatctgctgaacgactataggaaaatcgcttcaaaactgagcaaggtgcaggtctcaaacccacagttgaatccatataaggatatctttcaggaaaagtatgggttggacaaggatgcttcaggcatctacagtgtcaatatcaacaaattcgacgacatcttgaagaaactgtatagctttacggagttcgatctggcgactaagttccaagtgaaatgccgggagacatacatcggtcaatataaatattttaaactgtccaaccttctcaatgatagcatctacaatatcagtgaaggatataacattaataacctgaaagtgaatttccgaggccagaacgccaatttgaacccccggattatcaagcccattacaggacgggggctggtgaagaaaattattcgcttttgtaagaatatcgtgtcagtgaagggaataagaaagtag

SEQ ID NO: 18 - protein, 442 aa, bacteria
MHHHHHHPVVINSFNYNDPVNDDTILYMQIPYEEKSKKYYKAFEIMRNVWIIPERNTIGTDPSDFDPPASLENGSSAYYDPNYLTTDAEKDRYLKTTIKLFKRINSNPAGEVLLQEISYAKPYLGNEHTPINEFHPVTRTTSVNIKSSTNVKSSIILNLLVLGAGPDIFENSSYPVRKLMDSGGVYDPSNDGFGSINIVTFSPEYEYTFNDISGGYNSSTESFIADPAISLAHELIHALHGLYGARGVTYKETIKVKQAPLMIAEKPIRLEEFLTFGGQDLNIITSAMKEKIYNNLLANYEKIATRLSRVNSAPPEYDINEYKDYFQWKYGLDKNADGSYTVNENKFNEIYKKLYSFTEIDLANKFKVKCRNTYFIKYGFLKVPNLLDDDIYTVSEGFNIGNLAVNNRGQNIKLNPKIIDSIPDKGLVEKIVKFCKSVIPRK

SEQ ID NO: 19 - DNA, 1329 bp, bacteria
atgcaccatcatcatcaccatcccgtggttatcaatagctttaattataacgatcccgtgaatgatgatacaattctctacatgcagattccatacgaggaaaagagcaagaagtattataaagcattcgaaataatgcggaacgtttggattattcccgagagaaacacaatcggaaccgacccgtccgattttgatccacccgcctcattggaaaacggcagtagcgcctactacgatcccaattatctcaccacagatgctgagaaggaccgctatctgaaaaccacaatcaagctctttaagagaatcaactctaatccagctggcgaagtcctgctgcaggaaattagctacgcaaagccatatctcggcaacgagcatacacctattaatgagttccatcccgtcactcggacgacctctgtgaacataaaaagctctacaaacgtgaagagctctataatactgaacctgctcgtgctgggtgctggcccagacattttcgagaatagttcctatccagttcgaaagttgatggattctgggggcgtgtacgatcctagcaatgacggatttgggagtattaatatagtcacattcagtcccgagtatgaatacaccttcaacgacatcagcggtggctacaattcatcaactgagagcttcattgccgacccagccatcagtctggcccatgagttgatccatgccctgcacggcctctatggggctagaggggttacctacaaggaaacaattaaagtcaagcaggctccactcatgatcgctgaaaagcccattcggctcgaggagtttctgacattcggcggccaggatctcaacataatcaccagtgctatgaaagagaagatctacaataaccttcttgcaaattacgaaaaaatcgcaacacggctgtcacgggtgaatagcgctccccctgagtacgacattaacgagtataaagattacttccagtggaaatacgggctggacaaaaatgccgacgggagctacacagtgaacgagaacaagtttaacgagatctacaagaaactgtactcatttaccgagattgacctggctaataagtttaaggtcaagtgcagaaatacttatttcatcaagtacggatttttgaaagtccctaatctgctggacgacgatatttatactgtgtctgaaggttttaatatcggaaaccttgccgtgaataaccgcgggcagaatataaagcttaatcctaagatcatcgattcaattcctgacaaaggcctcgtcgagaaaatagtgaaattctgcaaaagtgtgattcctagaaagtga

SEQ ID NO: 20 - protein, 457 aa, bacteria
MPITINNFRYSDPVNNDTIIMMEPPYCKGLDIYYKAFKITDRIWIVPERYEFGTKPEDFNPPSSLIEGASEYYDPNYLRTDSDKDRFLQTMVKLFNRIKNNVAGEALLDKIINAIPYLGNSYSLLDKFDTNSNSVSFNLLEQDPSGATTKSAMLTNLIIFGPGPVLNKNEVRGIVLRVDNKNYFPCRDGFGSIMQMAFCPEYVPTFDNVIENITSLTIGKSKYFQDPALLLMHELIHVLHGLYGMQVSSHEIIPSKQEIYMQHTYPISAEELFTFGGQDANLISIDIKNDLYEKTLNDYKAIANKLSQVTSCNDPNIDIDSYKQIYQQKYQFDKDSNGQYIVNEDKFQILYNSIMYGFTEIELGKKFNIKTRLSYFSMNHDPVKIPNLLDDTIYNDTEGFNIESKDLKSEYKGQNMRVNTNAFRNVDGSGLVSKLIGLCKKIIPPTNIRENLYNRTA

SEQ ID NO: 21 - DNA, 1373 bp, bacteria
atgcccatcaccatcaacaacttccggtacagcgaccccgtgaacaacgacaccatcatcatgatggagcccccctactgcaagggcctggacatctactacaaggccttcaagatcaccgaccggatctggatcgtgcccgagcggtacgagttcggcaccaagcccgaggacttcaacccccccagcagcctgatcgagggcgccagcgagtactacgaccccaactacctgcggaccgacagcgacaaggaccggttcctgcagaccatggtgaagctgttcaaccggatcaagaacaacgtggccggcgaggccctgctggacaagatcatcaacgccatcccctacctgggcaacagctacagcctgctggacaagttcgacaccaacagcaacagcgtgagcttcaacctgctggagcaggaccccagcggcgccaccaccaagagcgccatgctgaccaacctgatcatcttcggccccggccccgtgctgaacaagaacgaggtgcggggcatcgtgctgcgggtggacaacaagaactacttcccctgccgggacggcttcggcagcatcatgcagatggccttctgccccgagtacgtgcccaccttcgacaacgtgatcgagaacatcaccagcctgaccatcggcaagagcaagtacttccaggaccccgccctgctgctgatgcacgagctgatccacgtgctgcacggcctgtacggcatgcaggtgagcagccacgagatcatccccagcaagcaggagatctacatgcagcacacctaccccatcagcgccgaggagctgttcaccttcggcggccaggacgccaacctgatcagcatcgacatcaagaacgacctgtacgagaagaccctgaacgactacaaggccatcgccaacaagctgagccaggtgaccagctgcaacgaccccaacatcgacatcgacagctacaagcagatctaccagcagaagtaccagttcgacaaggacagcaacggccagtacatcgtgaacgaggacaagttccagatcctgtacaacagcatcatgtacggcttcaccgagatcgagctgggcaagaagttcaacatcaagacccggctgagctacttcagcatgaaccacgaccccgtgaagatccccaacctgctggacgacaccatctacaacgacaccgagggcttcaacatcgagagcaaggacctgaagagcgagtacaagggccagaacatgcgggtgaacaccaacgccttccggaacgtggacggcagcggcctggtgagcaagctgatcggcctgtgcaagaagatcatcccccccaccaacatccgggagaacctgtacaaccggaccgcctg

SEQ ID NO: 22 - protein, 594 aa, human
MASSTPSSSATSSNAGADPNTTNLRPTTYDTWCGVAHGCTRKLGLKICGFLQRTNSLEEKSRLVSAFRERQSSKNLLSCENSDRDARFRRTETDFSNLFARDLLPAKNGEEQTVQFLLEVVDILLNYVRKTFDRSTKVLDFHHPHQLLEGMEGFNLELSDHPESLEQILVDCRDTLKYGVRTGHPRFFNQLSTGLDIIGLAGEWLTSTANTNMFTYEIAPVFVLMEQITLKKMREIVGWSSKDGDGIFSPGGAISNMYSIMAARYKYFPEVKTKGMAAVPKLVLFTSEQSHYSIKKAGAALGFGTDNVILIKCNERGKIIPADFEAKILEAKQKGYVPFYVNATAGTTVYGAFDPIQEIADICEKYNLWLHVDAAWGGGLLMSRKHRHKLNGIERANSVTWNPHKMMGVLLQCSAILVKEKGILQGCNQMCAGYLFQPDKQYDVSYDTGDKAIQCGRHVDIFKFWLMWKAKGTVGFENQINKCLELAEYLYAKIKNREEFEMVFNGEPEHTNVCFWYIPQSLRGVPDSPQRREKLHKVAPKIKALMMESGTTMVGYQPQGDKANFFRMVISNPAATQSDIDFLIEEIERLGQDL

SEQ ID NO: 23 - DNA, 1785 bp, human
atggcgtcttcgaccccatcttcgtccgcaacctcctcgaacgcgggagcggaccccaataccactaacctgcgccccacaacgtacgatacctggtgcggcgtggcccatggatgcaccagaaaactggggctcaagatctgcggcttcttgcaaaggaccaacagcctggaagagaagagtcgccttgtgagtgccttcagggagaggcaatcctccaagaacctgctttcctgtgaaaacagcgaccgggatgcccgcttccggcgcacagagactgacttctctaatctgtttgctagagatctgcttccggctaagaacggtgaggagcaaaccgtgcaattcctcctggaagtggtggacatactcctcaactatgtccgcaagacatttgatcgctccaccaaggtgctggactttcatcacccacaccagttgctggaaggcatggagggcttcaacttggagctctctgaccaccccgagtccctggagcagatcctggttgactgcagagacaccttgaagtatggggttcgcacaggtcatcctcgatttttcaaccagctctccactggattggatattattggcctagctggagaatggctgacatcaacggccaataccaacatgtttacatatgaaattgcaccagtgtttgtcctcatggaacaaataacacttaagaagatgagagagatagttggatggtcaagtaaagatggtgatgggatattttctcctgggggcgccatatccaacatgtacagcatcatggctgctcgctacaagtacttcccggaagttaagacaaagggcatggcggctgtgcctaaactggtcctcttcacctcagaacagagtcactattccataaagaaagctggggctgcacttggctttggaactgacaatgtgattttgataaagtgcaatgaaagggggaaaataattccagctgattttgaggcaaaaattcttgaagccaaacagaagggatatgttcccttttatgtcaatgcaactgctggcacgactgtttatggagcttttgatccgatacaagagattgcagatatatgtgagaaatataacctttggttgcatgtcgatgctgcctggggaggtgggctgctcatgtccaggaagcaccgccataaactcaacggcatagaaagggccaactcagtcacctggaaccctcacaagatgatgggcgtgctgttgcagtgctctgccattctcgtcaaggaaaagggtatactccaaggatgcaaccagatgtgtgcaggatatctcttccagccagacaagcagtatgatgtctcctacgacaccggggacaaggcaattcagtgtggccgccacgtggatatcttcaagttctggctgatgtggaaagcaaagggcacagtgggatttgaaaaccagatcaacaaatgcctggaactggctgaatacctctatgccaagattaaaaacagagaagaatttgagatggttttcaatggcgagcctgagcacacaaacgtctgtttttggtatattccacaaagcctcaggggtgtgccagacagccctcaacgacgggaaaagctacacaaggtggctccaaaaatcaaagccctgatgatggagtcaggtacgaccatggttggctaccagccccaaggggacaaggccaacttcttccggatggtcatctccaacccagccgctacccagtctgacattgacttcctcattgaggagatagaaagactgggccaggatctgtaa

SEQ ID NO: 24 - protein, 254 aa, plant
MVTSITLDLVNPTAGQYSSFVDKIRNNVKDPNLKYGGTDIAVIGPPSKEKFLRINFQSSRGTVSLGLKRDNLYVVAYLAMDNTNVNRAYYFRSEITSAESTALFPEATTANQKALEYTEDYQSIEKNAQITQGDQSRKELGLGIDLLSTSMEAVNKKARVVKDEARFLLIAIQMTAEAARFRYIQNLVIKNFPNKFNSENKVIQFEVNWKKISTAIYGDAKNGVFNKDYDFGFGKVRQVKDLQMGLLMYLGKPK

SEQ ID NO: 25 - DNA, 765 bp, plant
atggtaacatcaattaccctcgaccttgtcaaccctaccgctggacaatactcatccttcgtagataaaataaggaacaatgtcaaagaccctaatctcaagtacggtggtacagatatcgctgtcatcggccctccctcaaaagaaaaattcctcaggataaactttcaatcttccaggggaacggtctcacttggacttaagagggataatctgtatgtggtggcttatttggcaatggataatactaacgtgaatcgcgcatattactttcggagtgaaataacaagtgcagagagcaccgcattgttccccgaagcgacaactgcgaaccagaaagccttggaatacacagaggactatcagtccatcgaaaagaacgcgcagataactcaaggagaccagagtaggaaagaactcggcctcggcatcgatctcttgagtaccagcatggaggccgtgaacaaaaaggctagggtagttaaagatgaagccaggttcctcctgatagctatacagatgaccgctgaggccgccaggtttaggtatatccaaaaccttgtgatcaagaattttcccaacaaattcaacagcgagaataaggtgatacagtttgaggtaaactggaaaaaaatcagcaccgctatttatggggacgcgaaaaacggagtattcaataaagactacgatttcggcttcgggaaagttcgccaagttaaagacttgcaaatgggactgttgatgtatctcggcaaaccgaagtga

SEQ ID NO: 26 - protein, 217 aa, bacteria
MDIISVALKRHSTKAFDASKKLTPEQAEQIKTLLQYSPSSTNSQPWHFIVASTEEGKARVAKSAAGNYVFNERKMLDASHVVVFCAKTAMDDVWLKLVVDQEDADGRFATPEAKAANDKGRKFFADMHRKDLHDDAEWMAKQVYLNVGNFLLGVAALGLDAVPIEGFDAAILDAEFGLKEKGYTSLVVVPVGHHSVEDFNATLPKSRLPQNITLTEV

SEQ ID NO: 27 - DNA, 654 bp, bacteria
atggacataatttccgtcgctctcaagcgacattcaacaaaggcgtttgacgcttcaaaaaagttgacacctgaacaggcggaacagatcaagacgttgctccagtattccccgtcttctactaacagccagccctggcactttatcgtggcttccacagaggagggcaaagctcgagtagctaaaagcgcggcaggcaactatgtattcaatgagcgaaagatgcttgatgcgtcccatgtcgtggtattttgtgcgaagacagctatggacgatgtgtggcttaagctggtggtagatcaagaggatgccgacggcaggttcgccaccccagaagccaaggctgctaatgacaagggtcgcaaattttttgcggatatgcacaggaaagatctccacgacgatgccgaatggatggcaaaacaggtctacctcaacgtaggtaactttttgcttggtgtggctgctttgggtctggatgcggtgccgatcgagggctttgatgcggctatacttgatgctgagttcggcttgaaggaaaaaggatatacttcccttgtcgtagtgcccgttgggcatcatagtgtcgaggactttaacgctaccctgccgaaatctaggctcccgcaaaacataacactcacggaggtctga

SEQ ID NO: 28 - protein, 465 aa, bacteria
MHHHHHHQFVNKQFNYKDPVNGVDIAYIKIPNVGQMQPVKAFKIHNKIWVIPERDTFTNPEEGDLNPPPEAKQVPVSYYDSTYLSTDNEKDNYLKGVTKLFERIYSTDLGRMLLTSIVRGIPFWGGSTIDTELKVIDTNCINVIQPDGSYRSEELNLVIIGPSADIIQFECKSFGHEVLNLTRNGYGSTQYIRFSPDFTFGFEESLEVDTNPLLGAGKFATDPAVTLAHELIHAGHRLYGIAINPNRVFKVNTNAYYEMSGLEVSFEELRTFGGHDAKFIDSLQENEFRLYYYNKFKDIASTLNKAKSIVGTTASLQYMKNVFKEKYLLSEDTSGKFSVDKLKFDKLYKMLTEIYTEDNFVKFFKVLNRKTYLNFDKAVFKINIVPKVNYTIYDGFNLRNTNLAANFNGQNTEINNMNFTKLKNFTGLFEFYKLLCVRGIITSIMIIICCVILGIVIASTVGGIF

SEQ ID NO: 29 - DNA, 1401 bp, bacteria
atgcaccaccaccaccaccaccagttcgtgaataaacaattcaattataaagacccagtgaatggtgttgacatagcatacatcaaaatcccgaacgtgggacagatgcaaccggtgaaagccttcaagattcataacaagatctgggttattcctgaacgggacacttttaccaaccctgaagaaggtgacctgaaccctcctccagaggctaagcaggttcctgtttcctactacgattcaacttatctgagcactgataacgaaaaggataattaccttaagggagttaccaaactgttcgagcgcatttatagcacagacctcggcagaatgctgctgaccagcatagtgcggggaattccattttgggggggcagcacaatcgacacggagttgaaggtcatcgatacgaattgcatcaacgtgatacaaccagatggctcttacagatccgaggaactgaacctggtgatcatcggcccctctgctgatataatccaattcgaatgcaaaagcttcggtcacgaggtgctgaatcttacccggaacggatacgggtccacccagtacatacgctttagtcccgactttacattcggcttcgaggaaagtcttgaagtggacacgaatccactgctgggagctggcaagttcgccactgatcctgccgttacacttgctcatgaactgattcatgctggacaccggctttatgggatagctataaatccgaatagagtctttaaggttaacacaaatgcctactacgaaatgtctggccttgaggtttcattcgaggagcttaggacctttggaggccacgacgctaaattcatcgactctctgcaggagaatgagtttcggctgtactactacaacaagtttaaggacattgccagtactctgaacaaggctaagagcatcgtcgggaccacagccagcctccaatatatgaaaaacgtgttcaaggaaaagtaccttctgtcagaagacacatcaggaaaattctcagtcgacaaactgaaatttgacaagctgtacaagatgctgactgaaatatacacagaggacaacttcgtgaagttttttaaagtcctgaacagaaagacttacttgaacttcgacaaagccgtctttaaaatcaatatcgtcccaaaggttaattacactatctatgacggattcaatctcagaaacacgaacttggctgccaacttcaatggacagaacacagagatcaacaacatgaattttactaagcttaaaaatttcacaggcctgttcgagttctataagcttctttgcgtccgaggcatcattacatccatcatgatcataatctgctgtgtgatattgggcatagtgattgcatccaccgtggggggcatttttgcctag

SEQ ID NO: 30 - protein, 469 aa, bacteria
MHHHHHHPVTINNFNYNDPIDNNNIIMMEPPFARGTGRYYKAFKITDRIWIIPERYTFGYKPEDFNKSSGIFNRDVCEYYDPDYLNTNDKKNIFLQTMIKLFNRIKSKPLGEKLLEMIINGIPYLGDRRVPLEEFNTNIASVTVNKLISNPGEVERKKGIFANLIIFGPGPVLNENETIDIGIQNHFASREGFGGIMQMKFCPEYVSVFNNVQENKGASIFNRRGYFSDPALILMHELIHVLHGLYGIKVDDLPIVPNEKKFFMQSTDAIQAEELYTFGGQDPSIITPSTDKSIYDKVLQNFRGIVDRLNKVLVCISDPNININIYKNKFKDKYKFVEDSEGKYSIDVESFDKLYKSLMFGFTETNIAENYKIKTRASYFSDSLPPVKIKNLLDNEIYTIEEGFNISDKDMEKEYRGQNKAINKQAYEEISKEHLAVYKIQMCKSVIMIIICCVILGIVIASTVGGIFA

SEQ ID NO: 31 - DNA, 1410 bp, bacteria
atgcaccaccaccatcatcatcccgtgaccatcaacaatttcaactataatgaccctatcgataacaacaacatcattatgatggagccccctttcgcccgcggcaccgggagatactacaaggccttcaaaataaccgataggatctggatcatcccagagaggtacaccttcgggtacaagcctgaggactttaataaatcaagcggtatctttaatagggatgtgtgtgaatactacgaccctgactatctcaataccaacgacaaaaagaatatcttccttcagactatgatcaagcttttcaatcgaattaagagtaagccgcttggtgagaaactgctggagatgatcataaacggcatcccctacctcggagatcgccgcgttccgctggaagagtttaacactaatatcgcaagcgtcactgtaaataaactcatcagcaacccgggggaagtggaaaggaagaagggaatctttgctaacctgattatctttggaccaggcccagtgttgaatgaaaacgagaccatcgacatcgggatccagaaccactttgcatcacgagaggggtttggggggattatgcagatgaagttctgccccgagtacgtgtcagtgttcaataacgtgcaggaaaacaaaggagcatccatcttcaatcgccgaggctacttctctgatcctgctctcatcctcatgcacgagctcattcacgtgctgcacggactttatggcatcaaggtggacgacctgcctattgtgccgaatgaaaagaagttcttcatgcagagtactgatgccatccaggctgaggaactgtacactttcgggggccaggacccatccattatcaccccaagtactgataagtcaatctatgacaaagttctgcagaacttccgcggaatcgtggataggctcaacaaagtgctggtgtgtattagcgaccccaacattaacatcaatatttacaagaacaaattcaaggacaaatataaattcgtggaggactctgagggcaagtattcaattgacgtggagagcttcgacaaactgtacaaaagcctgatgttcggtttcacagagaccaacatagcagagaactataagattaaaactcgcgcgagctacttttcagattcactgcctccggtgaaaatcaagaacctcctggataatgagatctataccatagaagaaggatttaacatttccgacaaggacatggaaaaggagtaccggggacagaacaaggccatcaacaaacaggcctatgaagaaatcagcaaggagcacctcgccgtctacaaaattcaaatgtgcaaaagcgtcataatgattattatctgctgcgtaatcctggggatagtgatcgcttccaccgtaggcggcatcttcgcctga

SEQ ID NO: 32 - protein, 476 aa, bacteria
MHHHHHHPITINNFNYSDPVDNKNILYLDTHLNTLANEPEKAFRITGNIWVIPDRFSRNSNPNLNKPPRVTSPKSGYYDPNYLSTDSDKDPFLKEIIKLFKRINSREIGEELIYRLSTDIPFPGNNNTPINTFDFDVDFNSVDVKTRQGNNWVKTGSINPSVIITGPRENIIDPETSTFKLTNNTFAAQEGFGALSIISISPRFMLTYSNATNDVGEGRFSKSEFCMDPILILMHELNHAMHNLYGIAIPNDQTISSVTSNIFYSQYNVKLEYAEIYAFGGPTIDLIPKSARKYFEEKALDYYRSIAKRLNSITTANPSSFNKYIGEYKQKLIRKYRFVVESSGEVTVNRNKFVELYNELTQIFTEFNYAKIYNVQNRKIYLSNVYTPVTANILDDNVYDIQNGFNIPKSNLNVLFMGQNLSRNPALRKVNPENMLYLFTKFCHKAIDGRSLYNMMIILGVICAIILIIIIVYFST

SEQ ID NO: 33 - DNA, 1431 bp, bacteria
atgcaccaccatcatcatcatcctattacaatcaacaattttaattattctgacccagtggacaacaaaaacatactttaccttgatacccacctcaatactctggcgaacgagccagagaaagcgttccgcataacaggaaacatatgggtgattcctgacagattcagtcgaaatagtaacccaaacctgaacaagcctccgagggttacatcccctaagtccggttattacgaccccaattacctgtctacagatagcgataaagatcctttcctgaaagagatcattaaactgttcaaacgaataaactcccgcgaaatcggggaggaactcatttatcgattgtccacggacatccctttccctggtaataacaacaccccgattaatacctttgacttcgacgtcgactttaactctgtggatgtgaagactcggcagggtaacaactgggttaaaactgggtcaatcaacccgtctgtcataattacaggccctagggagaatataattgatccggagaccagcacctttaaattgactaataatactttcgccgcacaggaggggttcggcgccctgtctatcatatcaatcagtccccgatttatgctgacctactctaatgcaactaacgacgtcggggaaggtcggtttagcaaaagtgagttctgcatggacccgatcctcatactgatgcacgagttgaaccatgcaatgcataatctgtatggaatcgctattcccaacgatcagacaatatcttccgtcacgtcaaacattttctattctcagtataatgtgaaactggaatatgctgagatctacgcctttggtggccccacaattgacctgattccaaagagcgccaggaagtacttcgaggaaaaggcacttgattattataggagcatcgcaaagcgcctgaacagcatcacaacggccaacccaagctctttcaacaaatatataggcgaatacaagcaaaaactcattagaaaatacaggtttgtggtggaaagcagcggagaggtaaccgtaaaccgcaacaaattcgtggagctgtacaacgaactgactcagatctttacggaattcaattacgctaagatctacaatgtgcagaaccggaagatttacctgtccaatgtttacacacctgtcactgctaatattctcgatgacaatgtgtacgacattcagaatggcttcaacatccccaagtctaacctgaacgtgctgttcatgggccagaaccttagccgcaatcctgcgctgcgcaaagtcaaccctgagaatatgctgtatctcttcacgaagttctgtcacaaggccatagacggtagaagtctttataatatgatgattatactgggggtgatctgcgcgattatccttattattatcattgtatacttctctacatga